European Patent Specification EP 3 536 810 B1, published May 10, 2023. Title: COMPOSITIONS AND METHOD FOR DETECTING HUMAN PARVOVIRUS NUCLEIC ACID AND FOR DETECTING HEPATITIS A VIRUS NUCLEIC ACIDS IN SINGLE-PLEX OR MULTIPLEX ASSAYS. Applicant: Gen-Probe Incorporated Gao, Kui Norton, Kurt Craft Linnen, Jeffrey M. Gordon, Patricia C. Do, Dat Le, Tan N. The sequence listing filed with the application follows.

SEQUENCE LISTING (203 sequences)

SEQ ID NO: 1 - DNA, 20 bp, Artificial Sequence
  Synthetic Oligomer
cagagaattatgaaagtgga

SEQ ID NO: 2 - DNA, 23 bp, Artificial Sequence
  Synthetic Oligomer
agtcagagaattatgaaagtgga

SEQ ID NO: 3 - DNA, 27 bp, Artificial Sequence
  Synthetic Oligomer
ugagagtcagagaattatgaaagtgga

SEQ ID NO: 4 - DNA, 22 bp, Artificial Sequence
  Synthetic Oligomer
agtcagagaattatgaaagtgg

SEQ ID NO: 5 - DNA, 19 bp, Artificial Sequence
  Synthetic Oligomer
cagagaattatgaaagtgg

SEQ ID NO: 6 - DNA, 26 bp, Artificial Sequence
  Synthetic Oligomer
tgagagtcagagaattatgaaagtgg

SEQ ID NO: 7 - DNA, 18 bp, Artificial Sequence
  Synthetic Oligomer
tcagtgttcaatgaatgt

SEQ ID NO: 8 - DNA, 23 bp, Artificial Sequence
  Synthetic Oligomer
tttactcagtgttcaatgaatgt

SEQ ID NO: 9 - DNA, 27 bp, Artificial Sequence
  Synthetic Oligomer
ggagtttactcagtgttcaatgaatgt

SEQ ID NO: 10 - DNA, 35 bp, Artificial Sequence
  Synthetic Oligomer
atgaaagtggagtttactcagtgttcaatgaatgt

SEQ ID NO: 11 - DNA, 23 bp, Artificial Sequence
  Synthetic Oligomer
gaaagtcagagaataatgaaagt

SEQ ID NO: 12 - DNA, 56 bp, Artificial Sequence
  Synthetic Oligomer
aatttaatacgactcactatagggagaggaaaattaatcatggttttatcaatgtg

SEQ ID NO: 13 - DNA, 56 bp, Artificial Sequence
  Synthetic Oligomer
  misc_feature (48)..(48): N is inosine
aatttaatacgactcactatagggagaggaaaattaatcatggttttntcaatgtg

SEQ ID NO: 14 - DNA, 45 bp, Artificial Sequence
  Synthetic Oligomer
aatttaatacgactcactatagggagagcaggaaaattaatcatg

SEQ ID NO: 15 - DNA, 44 bp, Artificial Sequence
  Synthetic Oligomer
aatttaatacgactcactatagggagagcaggaaaattaatcat

SEQ ID NO: 16 - DNA, 43 bp, Artificial Sequence
  Synthetic Oligomer
aatttaatacgactcactatagggagagcaggaaaattaatca

SEQ ID NO: 17 - DNA, 42 bp, Artificial Sequence
  Synthetic Oligomer
aatttaatacgactcactatagggagagcaggaaaattaatc

SEQ ID NO: 18 - DNA, 54 bp, Artificial Sequence
  Synthetic Oligomer
aatttaatacgactcactatagggagaggcatagctgcaggaaaattaatcatg

SEQ ID NO: 19 - DNA, 53 bp, Artificial Sequence
  Synthetic Oligomer
aatttaatacgactcactatagggagaggcatagctgcaggaaaattaatcat

SEQ ID NO: 20 - DNA, 52 bp, Artificial Sequence
  Synthetic Oligomer
aatttaatacgactcactatagggagaggcatagctgcaggaaaattaatca

SEQ ID NO: 21 - DNA, 51 bp, Artificial Sequence
  Synthetic Oligomer
aatttaatacgactcactatagggagaggcatagctgcaggaaaattaatc

SEQ ID NO: 22 - DNA, 54 bp, Artificial Sequence
  Synthetic Oligomer
aatttaatacgactcactatagggagaactctttctaaaaagcgttttggagac

SEQ ID NO: 23 - DNA, 52 bp, Artificial Sequence
  Synthetic Oligomer
aatttaatacgactcactatagggagatctttctaaaaagcgttttggagac

SEQ ID NO: 24 - DNA, 54 bp, Artificial Sequence
  Synthetic Oligomer
aatttaatacgactcactatagggagaactctttctaaagagcgttttggagac

SEQ ID NO: 25 - DNA, 52 bp, Artificial Sequence
  Synthetic Oligomer
aatttaatacgactcactatagggagatctttctaaagagcgttttggagac

SEQ ID NO: 26 - DNA, 52 bp, Artificial Sequence
  Synthetic Oligomer
aatttaatacgactcactatagggagaactctttctaaaaagcgttttggag

SEQ ID NO: 27 - DNA, 52 bp, Artificial Sequence
  Synthetic Oligomer
aatttaatacgactcactatagggagaactctttctaaagagcgttttggag

SEQ ID NO: 28 - DNA, 55 bp, Artificial Sequence
  Synthetic Oligomer
aatttaatacgactcactatagggagaggaaaattaatcatggttttatcaatgt

SEQ ID NO: 29 - DNA, 29 bp, Artificial Sequence
  Synthetic Oligomer
ggaaaattaatcatggttttatcaatgtg

SEQ ID NO: 30 - DNA, 29 bp, Artificial Sequence
  Synthetic Oligomer
  misc_feature (21)..(21): N is inosine
ggaaaattaatcatggttttntcaatgtg

SEQ ID NO: 31 - DNA, 18 bp, Artificial Sequence
  Synthetic Oligomer
gcaggaaaattaatcatg

SEQ ID NO: 32 - DNA, 17 bp, Artificial Sequence
  Synthetic Oligomer
gcaggaaaattaatcat

SEQ ID NO: 33 - DNA, 16 bp, Artificial Sequence
  Synthetic Oligomer
gcaggaaaattaatca

SEQ ID NO: 34 - DNA, 15 bp, Artificial Sequence
  Synthetic Oligomer
gcaggaaaattaatc

SEQ ID NO: 35 - DNA, 27 bp, Artificial Sequence
  Synthetic Oligomer
ggcatagctgcaggaaaattaatcatg

SEQ ID NO: 36 - DNA, 26 bp, Artificial Sequence
  Synthetic Oligomer
ggcatagctgcaggaaaattaatcat

SEQ ID NO: 37 - DNA, 25 bp, Artificial Sequence
  Synthetic Oligomer
ggcatagctgcaggaaaattaatca

SEQ ID NO: 38 - DNA, 24 bp, Artificial Sequence
  Synthetic Oligomer
ggcatagctgcaggaaaattaatc

SEQ ID NO: 39 - DNA, 27 bp, Artificial Sequence
  Synthetic Oligomer
actctttctaaaaagcgttttggagac

SEQ ID NO: 40 - DNA, 25 bp, Artificial Sequence
  Synthetic Oligomer
tctttctaaaaagcgttttggagac

SEQ ID NO: 41 - DNA, 27 bp, Artificial Sequence
  Synthetic Oligomer
actctttctaaagagcgttttggagac

SEQ ID NO: 42 - DNA, 25 bp, Artificial Sequence
  Synthetic Oligomer
tctttctaaagagcgttttggagac

SEQ ID NO: 43 - DNA, 25 bp, Artificial Sequence
  Synthetic Oligomer
actctttctaaaaagcgttttggag

SEQ ID NO: 44 - DNA, 25 bp, Artificial Sequence
  Synthetic Oligomer
actctttctaaagagcgttttggag

SEQ ID NO: 45 - DNA, 28 bp, Artificial Sequence
  Synthetic Oligomer
ggaaaattaatcatggttttatcaatgt

SEQ ID NO: 46 - DNA, 59 bp, Artificial Sequence
  Synthetic Oligomer
ggucccucugaaauuaacauugguguuccaaaaaaaaaaaaaaaaaaaaaaaaaaaaaa

SEQ ID NO: 47 - DNA, 57 bp, Artificial Sequence
  Synthetic Oligomer
guuccaucauucuuuuuaugaacatttaaaaaaaaaaaaaaaaaaaaaaaaaaaaaa

SEQ ID NO: 48 - DNA, 62 bp, Artificial Sequence
  Synthetic Oligomer
ccuucgccuuuuccucuccaugccugauctttaaaaaaaaaaaaaaaaaaaaaaaaaaaaaa

SEQ ID NO: 49 - DNA, 59 bp, Artificial Sequence
  Synthetic Oligomer
ucgccuuuuccucuccaugccugauctttaaaaaaaaaaaaaaaaaaaaaaaaaaaaaa

SEQ ID NO: 50 - DNA, 59 bp, Artificial Sequence
  Synthetic Oligomer
ccuucgccuuuuccucuccaugccugtttaaaaaaaaaaaaaaaaaaaaaaaaaaaaaa

SEQ ID NO: 51 - DNA, 57 bp, Artificial Sequence
  Synthetic Oligomer
ggccccaccacacauuccaggaagtttaaaaaaaaaaaaaaaaaaaaaaaaaaaaaa

SEQ ID NO: 52 - DNA, 29 bp, Artificial Sequence
  Synthetic Oligomer
ggucccucugaaauuaacauugguguucc

SEQ ID NO: 53 - DNA, 24 bp, Artificial Sequence
  Synthetic Oligomer
guuccaucauucuuuuuaugaaca

SEQ ID NO: 54 - DNA, 29 bp, Artificial Sequence
  Synthetic Oligomer
ccuucgccuuuuccucuccaugccugauc

SEQ ID NO: 55 - DNA, 26 bp, Artificial Sequence
  Synthetic Oligomer
ucgccuuuuccucuccaugccugauc

SEQ ID NO: 56 - DNA, 26 bp, Artificial Sequence
  Synthetic Oligomer
ccuucgccuuuuccucuccaugccug

SEQ ID NO: 57 - DNA, 24 bp, Artificial Sequence
  Synthetic Oligomer
ggccccaccacacauuccaggaag

SEQ ID NO: 58 - DNA, 18 bp, Artificial Sequence
  Synthetic Oligomer
ucaguguucaaugaaugu

SEQ ID NO: 59 - DNA, 18 bp, Artificial Sequence
  Synthetic Oligomer
ucaguguucaaugaaugu

SEQ ID NO: 60 - DNA, 18 bp, Artificial Sequence
  Synthetic Oligomer
ucaguguucaaugaaugu

SEQ ID NO: 61 - DNA, 21 bp, Artificial Sequence
  Synthetic Oligomer
uguucaaugaauguggucucc

SEQ ID NO: 62 - DNA, 21 bp, Artificial Sequence
  Synthetic Oligomer
uguucaaugaauguggucucc

SEQ ID NO: 63 - DNA, 21 bp, Artificial Sequence
  Synthetic Oligomer
uguucaaugaauguggucucc

SEQ ID NO: 64 - DNA, 28 bp, Artificial Sequence
  Synthetic Oligomer
guucaaugaauguggucuccaaaacgcu

SEQ ID NO: 65 - DNA, 28 bp, Artificial Sequence
  Synthetic Oligomer
guucaaugaauguggucuccaaaacgcu

SEQ ID NO: 66 - DNA, 21 bp, Artificial Sequence
  Synthetic Oligomer
gaauguggucuccaaaacgcu

SEQ ID NO: 67 - DNA, 21 bp, Artificial Sequence
  Synthetic Oligomer
gaauguggucuccaaaacgct

SEQ ID NO: 68 - DNA, 21 bp, Artificial Sequence
  Synthetic Oligomer
gaauguggucuccaaaacgct

SEQ ID NO: 69 - DNA, 24 bp, Artificial Sequence
  Synthetic Oligomer
guggucuccaaaacgcuuuuuaga

SEQ ID NO: 70 - DNA, 24 bp, Artificial Sequence
  Synthetic Oligomer
guggucuccaaaacgcuuuuuaga

SEQ ID NO: 71 - DNA, 24 bp, Artificial Sequence
  Synthetic Oligomer
guggucuccaaaacgcuuuuuaga

SEQ ID NO: 72 - DNA, 24 bp, Artificial Sequence
  Synthetic Oligomer
guggucuccaaaacgcuuuuuaga

SEQ ID NO: 73 - DNA, 24 bp, Artificial Sequence
  Synthetic Oligomer
guggucuccaaaacgcuuuuuaga

SEQ ID NO: 74 - DNA, 20 bp, Artificial Sequence
  Synthetic Oligomer
gucuccaaaacgcuuuuuag

SEQ ID NO: 75 - DNA, 13 bp, Artificial Sequence
  Synthetic Oligomer
  misc_feature (7)..(7): N is G or Inosine
  misc_feature (12)..(12): N is G or Inosine
ccagtancagtna

SEQ ID NO: 76 - DNA, 16 bp, Artificial Sequence
  Synthetic Oligomer
tcatccagtagcagtg

SEQ ID NO: 77 - DNA, 14 bp, Artificial Sequence
  Synthetic Oligomer
tcacccagtaacag

SEQ ID NO: 78 - DNA, 24 bp, Artificial Sequence
  Synthetic Oligomer
tctgaccacccccatgccttatca

SEQ ID NO: 79 - DNA, 23 bp, Artificial Sequence
  Synthetic Oligomer
ctgaccacccccatgccttatca

SEQ ID NO: 80 - DNA, 19 bp, Artificial Sequence
  Synthetic Oligomer
ccacccccatgccttatca

SEQ ID NO: 81 - DNA, 24 bp, Artificial Sequence
  Synthetic Oligomer
ggacagttatctgaccacccccat

SEQ ID NO: 82 - DNA, 22 bp, Artificial Sequence
  Synthetic Oligomer
catggacagttatctgaccacc

SEQ ID NO: 83 - DNA, 24 bp, Artificial Sequence
  Synthetic Oligomer
catcattttcaaagtcatggacag

SEQ ID NO: 84 - DNA, 24 bp, Artificial Sequence
  Synthetic Oligomer
catcattttcagagtcatggacag

SEQ ID NO: 85 - DNA, 22 bp, Artificial Sequence
  Synthetic Oligomer
ctctccagacttatatagtcat

SEQ ID NO: 86 - DNA, 24 bp, Artificial Sequence
  Synthetic Oligomer
cctctctgtttgacttagttgctc

SEQ ID NO: 87 - DNA, 24 bp, Artificial Sequence
  Synthetic Oligomer
cctctttgtttgacttagttgctc

SEQ ID NO: 88 - DNA, 49 bp, Artificial Sequence
  Synthetic Oligomer
aatttaatacgactcactatagggagagctaacttgcccaggcttgtgt

SEQ ID NO: 89 - DNA, 51 bp, Artificial Sequence
  Synthetic Oligomer
aatttaatacgactcactatagggagaacgctaacttgcccaggcttgtgt

SEQ ID NO: 90 - DNA, 56 bp, Artificial Sequence
  Synthetic Oligomer
aatttaatacgactcactatagggagagttgtacgctaacttgcccaggcttgtgt

SEQ ID NO: 91 - DNA, 48 bp, Artificial Sequence
  Synthetic Oligomer
aatttaatacgactcactatagggagagctaacttgcccaggcttgtg

SEQ ID NO: 92 - DNA, 50 bp, Artificial Sequence
  Synthetic Oligomer
aatttaatacgactcactatagggagaacgctaacttgcccaggcttgtg

SEQ ID NO: 93 - DNA, 55 bp, Artificial Sequence
  Synthetic Oligomer
aatttaatacgactcactatagggagagttgtacgctaacttgcccaggcttgtg

SEQ ID NO: 94 - DNA, 47 bp, Artificial Sequence
  Synthetic Oligomer
aatttaatacgactcactatagggagaaacatagttagtaccgggta

SEQ ID NO: 95 - DNA, 48 bp, Artificial Sequence
  Synthetic Oligomer
aatttaatacgactcactatagggagacaacatagttagtaccgggta

SEQ ID NO: 96 - DNA, 49 bp, Artificial Sequence
  Synthetic Oligomer
aatttaatacgactcactatagggagaccaacatagttagtaccgggta

SEQ ID NO: 97 - DNA, 46 bp, Artificial Sequence
  Synthetic Oligomer
aatttaatacgactcactatagggagatgcgggggcccagcttgta

SEQ ID NO: 98 - DNA, 46 bp, Artificial Sequence
  Synthetic Oligomer
aatttaatacgactcactatagggagaggctatacctaaagtcatg

SEQ ID NO: 99 - DNA, 47 bp, Artificial Sequence
  Synthetic Oligomer
aatttaatacgactcactatagggagaggctatacctaaagtcatga

SEQ ID NO: 100 - DNA, 46 bp, Artificial Sequence
  Synthetic Oligomer
aatttaatacgactcactatagggagagctatacctaaagtcatga

SEQ ID NO: 101 - DNA, 51 bp, Artificial Sequence
  Synthetic Oligomer
aatttaatacgactcactatagggagaacctaaagtcatgaatccttgcag

SEQ ID NO: 102 - DNA, 50 bp, Artificial Sequence
  Synthetic Oligomer
aatttaatacgactcactatagggagaccaacatagttagtaccgggggt

SEQ ID NO: 103 - DNA, 49 bp, Artificial Sequence
  Synthetic Oligomer
aatttaatacgactcactatagggagaccaacatagttagtaccggggg

SEQ ID NO: 104 - DNA, 48 bp, Artificial Sequence
  Synthetic Oligomer
aatttaatacgactcactatagggagaccaacatagttagtaccgggg

SEQ ID NO: 105 - DNA, 47 bp, Artificial Sequence
  Synthetic Oligomer
aatttaatacgactcactatagggagaccaacatagttagtaccggg

SEQ ID NO: 106 - DNA, 46 bp, Artificial Sequence
  Synthetic Oligomer
aatttaatacgactcactatagggagaccaacatagttagtaccgg

SEQ ID NO: 107 - DNA, 45 bp, Artificial Sequence
  Synthetic Oligomer
aatttaatacgactcactatagggagaccaacatagttagtaccg

SEQ ID NO: 108 - DNA, 22 bp, Artificial Sequence
  Synthetic Oligomer
gctaacttgcccaggcttgtgt

SEQ ID NO: 109 - DNA, 24 bp, Artificial Sequence
  Synthetic Oligomer
acgctaacttgcccaggcttgtgt

SEQ ID NO: 110 - DNA, 29 bp, Artificial Sequence
  Synthetic Oligomer
gttgtacgctaacttgcccaggcttgtgt

SEQ ID NO: 111 - DNA, 21 bp, Artificial Sequence
  Synthetic Oligomer
gctaacttgcccaggcttgtg

SEQ ID NO: 112 - DNA, 23 bp, Artificial Sequence
  Synthetic Oligomer
acgctaacttgcccaggcttgtg

SEQ ID NO: 113 - DNA, 28 bp, Artificial Sequence
  Synthetic Oligomer
gttgtacgctaacttgcccaggcttgtg

SEQ ID NO: 114 - DNA, 20 bp, Artificial Sequence
  Synthetic Oligomer
aacatagttagtaccgggta

SEQ ID NO: 115 - DNA, 21 bp, Artificial Sequence
  Synthetic Oligomer
caacatagttagtaccgggta

SEQ ID NO: 116 - DNA, 22 bp, Artificial Sequence
  Synthetic Oligomer
ccaacatagttagtaccgggta

SEQ ID NO: 117 - DNA, 10 bp, Artificial Sequence
  Synthetic Oligomer
  misc_feature (7)..(7): N is G or Inosine
ccagtancag

SEQ ID NO: 118 - DNA, 19 bp, Artificial Sequence
  Synthetic Oligomer
ggctatacctaaagtcatg

SEQ ID NO: 119 - DNA, 20 bp, Artificial Sequence
  Synthetic Oligomer
ggctatacctaaagtcatga

SEQ ID NO: 120 - DNA, 19 bp, Artificial Sequence
  Synthetic Oligomer
gctatacctaaagtcatga

SEQ ID NO: 121 - DNA, 24 bp, Artificial Sequence
  Synthetic Oligomer
acctaaagtcatgaatccttgcag

SEQ ID NO: 122 - DNA, 23 bp, Artificial Sequence
  Synthetic Oligomer
ccaacatagttagtaccgggggt

SEQ ID NO: 123 - DNA, 22 bp, Artificial Sequence
  Synthetic Oligomer
ccaacatagttagtaccggggg

SEQ ID NO: 124 - DNA, 21 bp, Artificial Sequence
  Synthetic Oligomer
ccaacatagttagtaccgggg

SEQ ID NO: 125 - DNA, 20 bp, Artificial Sequence
  Synthetic Oligomer
ccaacatagttagtaccggg

SEQ ID NO: 126 - DNA, 19 bp, Artificial Sequence
  Synthetic Oligomer
ccaacatagttagtaccgg

SEQ ID NO: 127 - DNA, 18 bp, Artificial Sequence
  Synthetic Oligomer
ccaacatagttagtaccg

SEQ ID NO: 128 - DNA, 60 bp, Artificial Sequence
  Synthetic Oligomer
atgcgagcaactaagtcaaacagggagtttaaaaaaaaaaaaaaaaaaaaaaaaaaaaaa

SEQ ID NO: 129 - DNA, 52 bp, Artificial Sequence
  Synthetic Oligomer
tgcgggggcccagcttgtatttaaaaaaaaaaaaaaaaaaaaaaaaaaaaaa

SEQ ID NO: 130 - DNA, 59 bp, Artificial Sequence
  Synthetic Oligomer
tggctatacctaaagtcatgaatccttttaaaaaaaaaaaaaaaaaaaaaaaaaaaaaa

SEQ ID NO: 131 - DNA, 56 bp, Artificial Sequence
  Synthetic Oligomer
agtactgaaatccatatcggttgtttaaaaaaaaaaaaaaaaaaaaaaaaaaaaaa

SEQ ID NO: 132 - DNA, 27 bp, Artificial Sequence
  Synthetic Oligomer
atgcgagcaactaagtcaaacagggag

SEQ ID NO: 133 - DNA, 19 bp, Artificial Sequence
  Synthetic Oligomer
tgcgggggcccagcttgta

SEQ ID NO: 134 - DNA, 26 bp, Artificial Sequence
  Synthetic Oligomer
tggctatacctaaagtcatgaatcct

SEQ ID NO: 135 - DNA, 23 bp, Artificial Sequence
  Synthetic Oligomer
agtactgaaatccatatcggttg

SEQ ID NO: 136 - DNA, 21 bp, Artificial Sequence
  Synthetic Oligomer
gagtatatgggtttattccca

SEQ ID NO: 137 - DNA, 23 bp, Artificial Sequence
  Synthetic Oligomer
uacagaaccuagaggagaaaaug

SEQ ID NO: 138 - DNA, 19 bp, Artificial Sequence
  Synthetic Oligomer
uacagaaccuagaggagaa

SEQ ID NO: 139 - DNA, 19 bp, Artificial Sequence
  Synthetic Oligomer
gaaccuagaggagaaaaug

SEQ ID NO: 140 - DNA, 17 bp, Artificial Sequence
  Synthetic Oligomer
cagaaccuagaggagaa

SEQ ID NO: 141 - DNA, 21 bp, Artificial Sequence
  Synthetic Oligomer
cagaaccuagaggagaaaaug

SEQ ID NO: 142 - DNA, 21 bp, Artificial Sequence
  Synthetic Oligomer
cgugcagaaccuagaggagaa

SEQ ID NO: 143 - DNA, 21 bp, Artificial Sequence
  Synthetic Oligomer
cauacagaaccuagaggagaa

SEQ ID NO: 144 - DNA, 21 bp, Artificial Sequence
  Synthetic Oligomer
aguacagaaccuagaggagaa

SEQ ID NO: 145 - DNA, 19 bp, Artificial Sequence
  Synthetic Oligomer
uacagaaccuagaggagaa

SEQ ID NO: 146 - DNA, 19 bp, Artificial Sequence
  Synthetic Oligomer
ugcagaaccuagaggagaa

SEQ ID NO: 147 - DNA, 21 bp, Artificial Sequence
  Synthetic Oligomer
agugcagaaccuagaggagaa

SEQ ID NO: 148 - DNA, 17 bp, Artificial Sequence
  Synthetic Oligomer
cagaaccuagaggagaa

SEQ ID NO: 149 - DNA, 17 bp, Artificial Sequence
  Synthetic Oligomer
cagaaccuagaggagaa

SEQ ID NO: 150 - DNA, 21 bp, Artificial Sequence
  Synthetic Oligomer
cgugcagaaccuagaggagaa

SEQ ID NO: 151 - DNA, 21 bp, Artificial Sequence
  Synthetic Oligomer
cgugcagaaccuagaggagaa

SEQ ID NO: 152 - DNA, 21 bp, Artificial Sequence
  Synthetic Oligomer
cgugcagaaccuagaggagaa

SEQ ID NO: 153 - DNA, 21 bp, Artificial Sequence
  Synthetic Oligomer
cgugcagaaccuagaggagaa

SEQ ID NO: 154 - DNA, 21 bp, Artificial Sequence
  Synthetic Oligomer
cgugcagaaccuagaggagaa

SEQ ID NO: 155 - DNA, 21 bp, Artificial Sequence
  Synthetic Oligomer
cguacagaaccuagaggagaa

SEQ ID NO: 156 - DNA, 24 bp, Artificial Sequence
  Synthetic Oligomer
cgugcagaaccuagaggaggagau

SEQ ID NO: 157 - DNA, 20 bp, Artificial Sequence
  Synthetic Oligomer
gugcagaaccuagaggagaa

SEQ ID NO: 158 - DNA, 19 bp, Artificial Sequence
  Synthetic Oligomer
ugcagaaccuagaggagaa

SEQ ID NO: 159 - DNA, 19 bp, Artificial Sequence
  Synthetic Oligomer
gaaccuagaggagaagaug

SEQ ID NO: 160 - DNA, 21 bp, Artificial Sequence
  Synthetic Oligomer
caugcagaaccuagaggagaa

SEQ ID NO: 161 - DNA, 21 bp, Artificial Sequence
  Synthetic Oligomer
caugcagaaccuagaggagaa

SEQ ID NO: 162 - DNA, 22 bp, Artificial Sequence
  Synthetic Oligomer
gcagaaccuagaggagaaaaug

SEQ ID NO: 163 - DNA, 19 bp, Artificial Sequence
  Synthetic Oligomer
gaaccuagaggagaaaaug

SEQ ID NO: 164 - DNA, 19 bp, Artificial Sequence
  Synthetic Oligomer
gaacuuagaggagaaaaug

SEQ ID NO: 165 - DNA, 17 bp, Artificial Sequence
  Synthetic Oligomer
cagaaccuagaggagaa

SEQ ID NO: 166 - DNA, 17 bp, Artificial Sequence
  Synthetic Oligomer
cagaaccuagaggagaa

SEQ ID NO: 167 - DNA, 17 bp, Artificial Sequence
  Synthetic Oligomer
cagaaccuagaggagaa

SEQ ID NO: 168 - DNA, 19 bp, Artificial Sequence
  Synthetic Oligomer
gaaccuagaggagaaaaug

SEQ ID NO: 169 - DNA, 22 bp, Artificial Sequence
  Synthetic Oligomer
guauuaucuagugaagacuuac

SEQ ID NO: 170 - DNA, 17 bp, Artificial Sequence
  Synthetic Oligomer
cagagaatwatgaaagt

SEQ ID NO: 171 - DNA, 19 bp, Artificial Sequence
  Synthetic Oligomer
cagagaatwatgaaagtgg

SEQ ID NO: 172 - DNA, 27 bp, Artificial Sequence
  Synthetic Oligomer
tgaragtcagagaatwatgaaagtgga

SEQ ID NO: 173 - DNA, 12 bp, Artificial Sequence
  Synthetic Oligomer
gaatwatgaaag

SEQ ID NO: 174 - DNA, 39 bp, Artificial Sequence
  Synthetic Oligomer
gaaaattgaragtcagagaatwatgaaagtggarttyac

SEQ ID NO: 175 - DNA, 12 bp, Artificial Sequence
  Synthetic Oligomer
ggaaaattaatc

SEQ ID NO: 176 - DNA, 41 bp, Artificial Sequence
  Synthetic Oligomer
  misc_feature (33)..(33): N is A or Inosine
ggcatagctgcaggaaaattaatcatggttttntcaatgtg

SEQ ID NO: 177 - DNA, 53 bp, Artificial Sequence
  Synthetic Oligomer
  misc_feature (39)..(39): N is A or Inosine
gaaaaaggcatagctgcaggaaaattaatcatggttttntcaatgtgatgatg

SEQ ID NO: 178 - DNA, 40 bp, Artificial Sequence
  Synthetic Oligomer
tcagtgttcaatgaatgtggtctccaaaacgctttttaga

SEQ ID NO: 179 - DNA, 10 bp, Artificial Sequence
  Synthetic Oligomer
ccacccccat

SEQ ID NO: 180 - skipped

SEQ ID NO: 181 - DNA, 65 bp, Artificial Sequence
  Synthetic Oligomer
catcattttcaragtcatggacagttatctgaccacccccatgccttatcatccagtagcagtca

SEQ ID NO: 182 - DNA, 38 bp, Artificial Sequence
  Synthetic Oligomer
tctgaccacccccatgccttatcatccagtagcagtca

SEQ ID NO: 183 - DNA, 19 bp, Artificial Sequence
  Synthetic Oligomer
ccacccccatgccttatca

SEQ ID NO: 184 - DNA, 42 bp, Artificial Sequence
  Synthetic Oligomer
catcattttcaragtcatggacagttatctgaccacccccat

SEQ ID NO: 185 - DNA, 37 bp, Artificial Sequence
  Synthetic Oligomer
catcattttcaragtcatggacagttatctgaccacc

SEQ ID NO: 186 - DNA, 21 bp, Artificial Sequence
  Synthetic Oligomer
gctaacttgcccaggcttgtg

SEQ ID NO: 187 - DNA, 29 bp, Artificial Sequence
  Synthetic Oligomer
gttgtacgctaacttgcccaggcttgtgt

SEQ ID NO: 188 - DNA, 11 bp, Artificial Sequence
  Synthetic Oligomer
cttgcccaggc

SEQ ID NO: 189 - DNA, 39 bp, Artificial Sequence
  Synthetic Oligomer
gggtagttgtacgctaacttgcccaggcttgtgtaagtc

SEQ ID NO: 190 - DNA, 13 bp, Artificial Sequence
  Synthetic Oligomer
acctaaagtcatg

SEQ ID NO: 191 - DNA, 30 bp, Artificial Sequence
  Synthetic Oligomer
ggctatacctaaagtcatgaatccttgcag

SEQ ID NO: 192 - skipped

SEQ ID NO: 193 - DNA, 40 bp, Artificial Sequence
  Synthetic Oligomer
cagttggctatacctaaagtcatgaatccttgcagcactg

SEQ ID NO: 194 - DNA, 49 bp, Artificial Sequence
  Synthetic Oligomer
mrtrcagaacytagaggagaaratgcagtattatctagtgaagacttac

SEQ ID NO: 195 - DNA, 25 bp, Artificial Sequence
  Synthetic Oligomer
mrtrcagaacytagaggagaaratg

SEQ ID NO: 196 - DNA, 27 bp, Artificial Sequence
  Synthetic Oligomer
aatttaatacgactcactatagggaga

SEQ ID NO: 197 - DNA, 29 bp, Artificial Sequence
  Synthetic Oligomer
cttatcacacaagcctgggcaagttagct

SEQ ID NO: 198 - DNA, 7477 bp, Hepatitis A virus
  ref <308>: GenBank / AB020564.1  GI:4001732
  ref <309>: 2001-08-04
  ref <313>: (1)..(7477)
ttcaagaggggtctccggagttttccggagcccctcttggaagtccatggtgaggggacttgatacctcaccgccgtttgcctaggctataggctaaatttccctttccctgtccttcccctattcccctttgttttgtttgtaaatattaattcctgcaggttcagggttctttaatctgtttctctataagaacactcaattttcacgctttctgtcttctttcttccagggctctccccttgccctaggctctggccgttgcgcccggcggggtcaactccatgattagcatggagctgtaggagtctaaattggggacgcagatgtttgggacgtcaccttgcagtgttaacttggctttcatgaacctctttgatctttcacaagaggtaggctacgggtgaaacctcttaggctaatacttctatgaagagatgccttggatagggtaacagcggcggatattggtgagttgttaagacaaaaaccattcaacgccgaaggactggttctcatccagtggatgcattgagtgaattgattgtcaaggctgtctctaggtttaatcccagacctctctgtgcttagggcaaacactatttggccttaaatgggatcctgtgagagggggtccctccattgacagctggactgttctttggggccttatgtggtgtttgcctctgaggtactcaggggcatttaggtttttcctcattcttaaacaataatgaatatgtccaaacaaggaattttccagactgttgggagtggccttgaccacatcctgtctctggcagatattgaggaagaacaaatgattcagtccgttgataggactgcagtgactggtgcttcttattttacttctgtggaccaatcgtcagttcacactgctgaggttggctcacatcaaattgaacctttgaaaacctctgttgataaacctggttctaagaagactcagggggagaagtttttcttgattcactctgctgattggcttactacacatgctctttttcatgaagttgcaaaattggatgtggtgaaattactgtataatgagcaatttgctgtccaaggcttgttgagatatcacacatatgcaagatttggcattgagattcaagttcagataaaccctacaccctttcagcaagggggattaatttgtgccatggttcctggtgaccaaagttatggttcaatagcatccttgactgtttatcctcatggtctgttaaattgtaacatcaacaatgttgttagaataaaggttccattcatttatactagaggtgcttatcattttaaagatccacagtacccagtttgggaattaacaatcagagtttggtcagagttgaatattggaacaggaacttcggcttacacttcacttaacgttttagctaggtttacagatttggagttacatggtttaactcctctttctacacagatgatgagaaatgaatttagagttagtactactgaaaatgttgtaaacttgtcaaattatgaagatgcaagggcaaaaatgtcttttgctttggatcaggaagattggaagtctgatccctctcaaggtggtggaattaaaattactcattttactacttggacatccattccaaccttagctgcccagtttccgtttaatgcttcagattcggttgggcaacaaattaaagttattccagtggacccatattttttccagatgacaaacactaatcctgaccaaaaatgtataactgccctggcttctatttgtcagatgttttgtttttggaggggagatcttgtttttgattttcaggtttttccaactaaatatcattcaggtagattattgttttgttttgttcctgggaatgagttaatagatgttactggaattacattaaagcaggcaactactgctccttgtgcagtgatggacattacaggagtgcaatcaactttgagatttcgtgttccttggatttctgatacaccctatcgagtaaataggtacacgaagtcggcacatcaaaaaggtgagtacactgccattggaaagcttattgtgtactgttacaatagactgacttctccttctaatgttgcttctcatgttagagttaatgtttatctttcagcaattaatctggaatgttttgctcctctttatcatgctatggatgttaccacacaagttggagatgattcaggaggtttttcaacaacagtttctactgagcagaatgttcctgatccccaagttggcataacaaccatgagggacctaaaagggaaagccaatagaggaaagatggatgtttcaggtgtgcaagcacctgtgggagctatcacaacaattgaggatccagttttagcaaagaaagtgcctgagacatttcctgaattgaaacctggagagtctagacatacatcagatcatatgtctatttataaatttatgggaaggtctcattttctgtgtacttttacttttaattcaaataataaagagtacacatttccaataactctgtcttcgacttctaatcctcctcatggtttaccatcaacattaaggtggttcttcaatctgtttcagttgtatagaggaccattggatttgacaattattatcacaggagccactgatgtggatggtatggcctggttcactccagtaggccttgctgtcgacaccccttgggtggaaaaggagtcagctttgtctattgattacaaaactgctcttggagctgttagatttaatacaagaagaacagggaatattcagattagattgccatggtattcttatttgtatgccgtgtctggagcactggatggtctgggggataaaacagattccacatttggattggtttccattcagattgcaaattacaatcattctgatgaatatttgtcctttagttgctatttgtctgttacagaacaatcagagttctattttcctagagctccattaaattcaaatgctatgttgtccactgagtccatgatgagcagaattgcagctggggacttggagtcatcggtggatgatcctagatcagaggaggacagaagatttgagagtcatatagaaagtaggaaaccatacaaagaattgagattggaggttggcaaacaaagactcaagtatgctcaggaagaactgtcaaatgaggtgcttccacctcctaggaaaataaaggggctattttcacaagctaaaatttctcttttttatactgaggagcatgaaataatgaaattttcttggagaggagtaactgctgacactagggctttgagaagatttggattctctatggctgctggtagaagtgtgtggactcttgagatggatgctggagttcttactggaagattggtcagattgaatgatgagaaatggacagaaatgaaagatgataaaattgtttcattaatcgaaaaattcacaagcaacaaatattggtctaaagtgaattttccacatggaatgttagatcttgaagaaattgctgccaactctaaagattttccaaatatgtctgagacagatttgtgtttcctgttgcattggctgaatccaaagaaaataaatttagcagatagaatgcttggattgtctggagtgcaggaaattaaagaacagggtgttggattgatagcagagtgtagaactttcttggattctattgctgggactctgaaatccatgatgtttggatttcatcattctgtgactgttgaaattataaatactgtgctttgttttgttaagagtggaattctactctatgtcatacaacaattgaaccaagatgagcactcccacataattggtttgttgagagtcatgaattatgcagatattggctgctcagttatttcatgtggcaaagttttttctaaaatgttagaaacagtttttaattggcaaatggactccagaatgatggagctgagaactcagagcttttccaattggctaagagacatttgttcaggaattactatttttaaaagttttaaggatgccatatattggttatatacaaaattgaaggatttttatgaagtaaattatggcaagaagaaggatgttcttaatattcttaaagataaccagcaaaaaatagaaaaagctattgaagaagcagacaatttttgcattttgcaaattcaagatgtagaaaaatttgatcagtatcagaaaggggttgatttaatacaaaagctgagaactgttcattcaatggctcaagttgaccctagccttggggttcatttgtcacctcttagagattgtatagccagagtccaccaaaagctcaagaatcttggatctataaatcaggccatggtgacaagtagtgagccagttgtttgctatttatatggcaaaagaggaggagggaaaagcttgacttcaattgcattggcaaccaagatttgtaaacactatggtgttgaacctgagaaaaatatttacactaaacctgtggcttcagactattgggatggttatagtggacaattggtttgcattattgatgatattggccaaaatacaacagatgaagattggtcagatttttgtcaattagtgtcaggatgcccaatgagattgaatatggcttctcttgaggagaagggcagacatttttcctctccttttataatagcaacttcaaattggtcaaatccaagtccaaaaacagtttatgttaaggaagcaattgatcgtaggcttcattttaaggttgaagttaaacctgcttcattttttaaaaatcctcataatgatatgttaaatgttaatttggctaaaacaaatgatgcaattaaggacatgtcttgtgttgatctagtaatggatggacataacatttcattgatggatttacttagttctttagtgatgacagttgaaattaggaagcaaaatatgagtgaattcatggagttgtggtcccagggaatctcagatgatgacaatgatagtgcagtagctgagtttttccaatcttttccatctggtgaaccatcaaattccaaattatctagttttttccaatctgtcactaatcacaagtgggttgctgtgggagctgcagttggcattcttggagtgcttgtgggaggatggttcgtgtacaagcatttctcccgcaaagaggaagaaccaattccagctgaaggggtttatcatggcgtgactaagcccaaacaggtgattaaattggatgcagatccagtagagtctcagtcaactttagaaatagcaggattagttaggaaaaatttggttcagtttggagttggggagaaaaatggatgtgtgagatgggttatgaatgccttgggagtgaaggatgattggttattagtaccttctcatgcttacaaatttgaaaaggattatgaaatgatggagttttatttcaatagaggtggaacttactattcaatttcagctggaaatgttgttattcaatctttagatgtggggtttcaagatgttgttctaatgaaggttcctacaattcccaagtttagagatattactcaacattttattaagaaaggagatgtacctagagccttgaatcgcttggcaacattagtgacaactgttaatggaactcctatgttaatttctgagggaccattaaagatggaggaaaaagccacttatgttcataagaagaatgatggtaccacagttgatttgactgttgatcaggcatggagaggaaaaggtgaaggtcttcctggaatgtgtggtggggctctggtgtcatcaaatcagtccatacagaatgcaattttgggtattcatgttgctggaggaaattcaattcttgtggcaaagttggttactcaagaaatgttccaaaatattgataagaaaattgaaagtcagagaataatgaaagtggaattcactcagtgttcaatgaatgtagtctccaaaacgctttttagaaagagtcccattcatcatcacattgataaaaccatgattaattttcctgcagctatgcctttttctaaagttgaaattgatccaatggctgtgatgttgtctaaatattcattacctcttgtagaagaaccagaggattacaaagaagcttcagttttttatcaaaacaagatagtaggcaagactcagttagttgatgactttttagatcttgatatggccattacaggggctccaggcattgatgctattaatatggattcatctcctgggtttccttatgttcaagaaaaattgactaaaagagatttaatttggttggatgaaaatggtttgctgctaggagttcatccaagattggctcagagaattttatttaacactgtcatgatggaaaattgttctgacctagatgttgtttttacaacttgtccaaaagatgaattgagacctttagagaaagttttggaatcaaaaacaagagcaattgatgcttgtcctttggattatacaattttatgtcgaatgtactggggtccagctattagttattttcatttgaatccagggtttcacacaggtgttgctattggcatagatcctgatagacagtgggatgaattatttaaaccaatgataagatttggagatgttggtcttgatttagatttttctgcctttgatgctagtcttagtccatttatgatcagggaggcgggtagaatcatgagtgaattatctggaacaccatctcattttggaacggctcttatcaatactatcatttattctaaacatttgctgtacaattgttgttatcatgtctgtggttcaatgccttctgggtccccttgtacagctttgttgaattcaattattaacaacattaatttgtattatgtgttttctaaaatatttggaaagtctccagttttcttttgtcaagctctgaggatcctttgttatggagatgatgttttgatagttttttccagagatgttcaaattgataatcttgatttgattggacagaaaattgtggatgaattcaaaaaacttggcatgacagccacttcagctgataaaaatgtgcctcaactgaagccagtttcagaattgacctttcttaaaagatcttttaatttggtggaggacagaattaggcctgcaatttcagaaaagacaatttggtctttgatagcttggcagagaagcaacgctgagtttgagcagaatttagaaaatgctcagtggtttgcttttatgcatggctatgagttttatcagaaattttattattttgttcagtcctgtttggagaaagagatgatagaatataggcttaaatcttatgattggtggagaatgagattttatgaccagtgtttcatttgtgacctttcatgatttgtttaaacaaattttcttaaaatttctgaggtttgtttatttcttttatcagtaaat

SEQ ID NO: 199 - DNA, 5594 bp, Erythrovirus B19
  ref <308>: GenBank / AF162273.1 GI:5670171
  ref <309>: 1999-08-02
  ref <313>: (1)..(5594)
ccaaatcagatgccgccggtcgccgccggtaggcgggacttccggtacaagatggcggacaattacgtcatttcctgtgacgtcatttcctgtgacgtcacttccggtgggcgggacttccggaattagggttggctctgggccagcttgcttggggttgccttgacactaagacaagcggcgcgccgcttgtcttagtggcacgtcaaccccaagcgctggcccagagccaaccctaattccggaagtcccgcccaccggaagtgacgtcacaggaaatgacgtcacaggaaatgacgtaattgtccgccatcttgtaccggaagtcccgcctaccggcggcgaccggcggcatctgatttggtgtcttcttttaaattttagcgggcttttttcccgccttatgcaaatgggcagccattttaagtgtttcactataattttattggtcagttttgtaacggttaaaatgggcggagcgtaggcggggactacagtatatatagcacggcactgccgcagctctttctttctgggctgctttttcctggactttcttgctgttttttgtgagctaactaacaggtatttatactacttgttaacatactaacatggagctatttagaggggtgcttcaagtttcttctaatgttctggactgtgctaacgataactggtggtgctctttactggatttagacacttctgactgggaaccactaactcatactaacagactaatggcaatatacttaagcagtgtggcttctaagcttgactttaccggggggccactagcggggtgcttgtacttttttcaagtagaatgtaacaaatttgaagaaggctatcatattcatgtggttattggggggccagggttaaaccccagaaacctcacagtgtgtgtagaggggttatttaataatgtactttatcaccttgtaactgaaaatgtaaagctaaaatttttgccaggaatgactacaaaaggcaaatactttagagatggagagcagtttatagaaaactatttaatgaaaaaaatacctttaaatgttgtatggtgtgttactaatattgatggatatatagatacctgtatttctgctacttttagaaggggagcttgccatgccaagaaaccccgcattaccacagccataaatgacactagtagtgatgctggggagtctagcggcacaggggcagaggttgtgccaattaatgggaagggaactaaggctagcataaagtttcaaactatggtaaactggttgtgtgaaaacagagtgtttacagaggataagtggaaactagttgactttaaccagtacactttactaagcagtagtcacagtggaagttttcaaattcaaagtgcactaaaactagcaatttataaagcaactaatttagtgcctacaagcacatttctattgcatacagactttgagcaggttatgtgtattaaagacaataaaattgttaaattgttactttgtcaaaactatgaccccctattagtggggcagcatgtgttaaagtggattgataaaaaatgtggcaagaaaaatacactgtggttttatgggccgccaagtacaggaaaaacaaacttggcaatggccattgctaaaagtgttccagtatatggcatggttaactggaataatgaaaactttccatttaatgatgtagcagggaaaagcttggtggtctgggatgaaggtattattaagtctacaattgtagaagctgcaaaagccattttaggcgggcaacccaccagggtagatcaaaaaatgcgtggaagtgtagctgtgcctggagtacctgtggttataaccagcaatggtgacattacttttgttgtaagcgggaacactacaacaactgtacatgctaaagccttaaaagagcgaatggtaaagttaaactttactgtaagatgcagccctgacatggggttactaacagaggctgatgtacaacagtggcttacatggtgtaatgcacaaagctgggaccactatgaaaactgggcaataaactacacttttgatttccctggaattaatgcagatgccctccacccagacctccaaaccaccccaattgtcacagacaccagtatcagcagcagtggtggtgaaagctctgaagaactcagtgaaagcagcttttttaacctcatcaccccaggcgcctggaacactgaaaccccgcgctctagtacgcccatccccgggaccagttcaggagaatcatttgtcggaagctcagtttcctccgaagttgtagctgcatcgtgggaagaagccttctacacacctttggcagaccagtttcgtgaactgttagttggggttgattatgtgtgggacggtgtaaggggtttacctgtgtgttgtgtgcaacatattaacaatagtgggggaggcttgggactttgtccccattgcattaatgtaggggcttggtataatggatggaaatttcgagaatttaccccagatttggtgcggtgtagctgccatgtgggagcttctaatcccttttctgtgctaacctgcaaaaaatgtgcttacctgtctggattgcaaagctttgtagattatgagtaaagaaagtggcaaatggtgggaaagtgatgataaatttgctaaagctgtgtatcagcaatttgtggaattttatgaaaaggttactggaacagacttagagcttattcaaatattaaaagatcactataatatttctttagataatcccctagaaaacccatcctctctgtttgacttagttgctcgtattaaaaataaccttaaaaactctccagacttatatagtcatcattttcaaagtcatggacagttatctgaccacccccatgccttatcatccagtagcagtcatgcagaacctagaggagaaaatgcagtattatctagtgaagacttacacaagcctgggcaagttagcgtacaactacccggtactaactatgttgggcctggcaatgagctacaagctgggcccccgcaaagtgctgttgacagtgctgcaaggattcatgactttaggtatagccaactggctaagttgggaataaatccatatactcattggactgtagcagatgaagagcttttaaaaaatataaaaaatgaaactgggtttcaagcacaagtagtaaaagactactttactttaaaaggtgcagctgcccctgtggcccattttcaaggaagtttgccggaagttcccgcttacaacgcctcagaaaaatacccaagcatgacttcagttaattctgcagaagccagcactggtgcaggagggggtggcagtaatcctgtcaaaagcatgtggagtgagggggccacttttagtgccaactctgtaacttgtacattttccagacagtttttaattccttatgacccagagcaccattataaggtgttttctcccgcagcaagcagctgccacaatgccagtggaaaggaggcaaaggtttgcacaattagtcccataatgggatactcaaccccatggagatatttagattttaatgctttaaatttatttttttcacctttagagtttcagcacttaattgaaaattatggaagtatagctcctgatgctttaactgtaaccatatcagaaattgctgttaaggatgttacagacaaaactggagggggggtacaggttactgacagcactacagggcgcctatccatgttagtagaccatgaatacaagtacccatatgtgttaggacaaggtcaggatactttagccccagaacttcctatttgggtatactttccccctcaatatgcttacttaacagtaggagatgttaacacacaaggaatctctggagacagcaaaaaattagcaagtgaagaatcagcattttatgttttggaacacagttcttttcagcttttaggtacaggaggtacagcaactatgtcttataagtttcctccagtgcccccagaaaatttagagggctgcagtcaacacttttatgaaatgtacaatcccttatacggatcccgcttaggggttcctgacacattaggaggtgacccaaaatttagatctttaacacatgaagaccatgcaattcagccccaaaacttcatgccagggccactagtaaactcagtgtctacaaaggagggagacagctctaatactggagctggaaaagccttaacaggccttagcacaggcacctctcaaaacactagaatatccttacgccctgggccagtgtcacagccataccaccactgggacacagataaatatgttccaggaataaatgccatttctcatggtcagaccacttatggtaacgctgaagacaaagagtatcagcaaggagtgggtagatttccaaatgaaaaagaacagctaaaacagttacagggtttaaacatgcacacctatttccccaataaaggaacccagcaatatacagatcaaattgagcgccccctaatggtgggttctgtatggaacagaagagcccttcactatgaaagccagctgtggagtaaaattccaaatttagatgacagttttaaaactcagtttgcagccttaggaggatggggtttgcatcagccacctcctcaaatatttttaaaaatattaccacaaagtgggccaattggaggtattaaatcaatgggaattactaccttagttcagtatgccgtgggaattatgacagtaactatgacatttaaattggggccccgtaaagctacgggacggtggaatcctcaacctggagtatatcccccgcacgcagcaggtcatttaccatatgtactatatgaccccacagctacagatgcaaaacaacaccacaggcatggatacgaaaagcctgaagaattgtggacagccaaaagccgtgtgcacccattgtaaacactccccaccgtgccctcagccaggatgcgtaactaaacgcccaccagtaccacccagactgtacctgccccctcctgtacctataagacagcctaacacaaaagatatagacaatgtagaatttaagtacttaaccagatatgaacaacatgttattagaatgttaagattgtgtaatatgtatcaaaatttagaaaaataaacatttgttgtggttaaaaaattatgttgttgcgctttaaaaatttaaaagaagacaccaaatcagatgccgccggtcgccgccggtaggcgggacttccggtacaagatggcggacaattacgtcatttcctgtgacgtcatttcctgtgacgtcacttccggtgggcgggacttccggaattagggttggctctgggccagcgcttggggttgacgtgccactaagacaagcggcgcgccgcttgtcttagtgtcaaggcaaccccaagcaagctggcccagagccaaccctaattccggaagtcccgcccaccggaagtgacgtcacaggaaatgacgtcacaggaaatgacgtaattgtccgccatcttgtaccggaagtcccgcctaccggcggcgaccggcggcatctgatttgg

SEQ ID NO: 200 - DNA, 472 bp, Artificial Sequence
  Synthetic Oligomer
aaatattaaaagatcattataatatttctttagataatcccctagaaaacccatcctctctgtttgacttagttgctcgtattaaaaataaccttaaaaactctccagacttatatagtcatcattttcaaagtcatggacagttatctgaccacccccatgccttatcatccagtagcagtcatgcagaacctagaggagaagatgcagtattatctagtgaagacttacacaagcctgggcaagttagcgtacaactacccggtactaactatgttgggcctggcaatgagctacaagctgggcccccgcaaagtgctgttgacagtgctgcaaggattcatgactttaggtatagccaactggctaagttgggaataaatccatatactcattggactgtagcagatgaagagcttttaaaaaatataaaaaatgaaaccgggtttcaagcacaagtagtaaaagacta

SEQ ID NO: 201 - DNA, 471 bp, Artificial Sequence
  Synthetic Oligomer
aatattaaaagatcattacaatatttctttagataatcccctagaaaacccatcttccctgtttgacttagttgctcgtattaaaagtaatcttaaagactctccagacctatatagtcatcattttcaaagtcatggacagttatctgaccacccccatgccttatcacccagtagcagtcatacagaacctagaggagaaaatgcagtattatctagtgaagacttacacaagcctgggcaagttagcatacaactacccggtactaactatgttgggcctggcaatgagctacaagctgggcccccgcaaagtgctgtggacagtgctgcaaggattcatgactttaggtatagccaattggctaagctgggaataaacccatatacttattggactgtagcagatgaggaactgttaaaaaatataaaaaatgaaactgggtttcaagcacaagcagtaaaagatta

SEQ ID NO: 202 - DNA, 472 bp, Artificial Sequence
  Synthetic Oligomer
aaattttaaaagatcattacaacatttctttagacaatcctttagaaaacccctcttctttatttgacttagttgctcgcattaaaagcaatcttaaaaactctccagacctatatagtcatcattttcagagccatggacagttatctgaccacccccattccttatcacccagtaacagtagtacagaacctagaggagaaaatgcagtattatctagtgaagacttacacaagcctgggcaagttagcatacaattacccggtactaactatgttgggcctggcaatgagctacaagctgggcctccgcagaatgctgtggacagtgctgcaaggattcatgactttaggtatagccaattggctaagttgggaataaatccttatactcattggacggtagcagatgaggaattgttaaaaaatataaaaaatgaaacagggtttcaagcacaagcagtaaaagacta

SEQ ID NO: 203 - DNA, 1039 bp, Artificial Sequence
  Synthetic Oligomer
tttgtcggaagcccagtttcctccgaagttgtagctgcatcgtgggaagaagccttctacacacctttggcagaccagtttcgtgaactgttagttggggttgattatgtgtgggacggtgtaaggggcttacctgtgtgttgtgtgcaacatattaacaatagtgggggaggcttgggactttgtccccattgcattaatgtaggggcttggtataatggatggaaatttcgagaatttactccagatttggtgcgatgtagctgccatgtgggagcttctaatcccttttctgtgctaacctgtaaaaaatgtgcttacctgtctggattgcaaagctttgtagattatgagtaaagaaagtggcaaatggtgggaaagtaatgataaatttgctaaagctgtgtatcagcaatttgtggaattttatgaaaaagttactggaacagacttagagcttattcaaatattaaaagaccattataatatttctttagataatcccctagaaaacccatcctctctgtttgacttagttgctcgtattaaaaataaccttaaaaactctccagacttatatagtcatcattttcaaagtcatggacagttatctgaccacccccatgccttatcatccagtagcagtcatgcagaacctagaggagaaaatgcagtattatctagtgaagacttacacaagcctgggcaagttagcgtacaactacccggtactaactatgttgggcctggcaatgagctacaagctgggcccccgcaaagtgctgttgacagtgctgcaaggattcatgactttaggtatagccaactggctaagttgggaataaatccatatactcattggactgtagcagatgaagagcttttaaaaaatataaaaaatgaaactgggtttcaagcacaagtagtaaaagactactttactttaaaaggtgcagctgcccctgtggcccattttcaaggaagtttgccggaagttcccgcttacaacgcctcagaaaaatacccaagcatgacttca